European Patent Specification EP 3 512 548 B1, published March 22, 2023. Title: Antibody and checkpoint inhibitor combination therapy. Applicant: Bionomics Limited. The sequence listing filed with the application follows.

SEQUENCE LISTING (10 sequences)

SEQ ID NO: 1 - protein, 24 aa, mus musculus
  misc_feature: Heavy Chain CDR1
GLYTYRTHRPHESERGLYTYRTRP

SEQ ID NO: 2 - protein, 22 aa, mus musculus
  MISC_FEATURE: 18G7.1 Heavy Chain CDR2 Amino Acid
ILELEPRGLYSERASPSERTHR

SEQ ID NO: 3 - protein, 33 aa, mus musculus
  MISC_FEATURE: Heavy Chain CDR3
ALAARGSERGLYTYRTYRGLYSERSERGLNTYR

SEQ ID NO: 4 - protein, 29 aa, mus musculus
  MISC_FEATURE: Light Chain CDR1
GLSERVALASPSERTYRGLYASNSERPHE

SEQ ID NO: 5 - protein, 8 aa, mus musculus
  MISC_FEATURE: Light Chain CDR2
LETHRSER

SEQ ID NO: 6 - protein, 25 aa, Artificial
  Synthetic
  MISC_FEATURE: Light Chain CDR3
GLNGLNASNALAGLASPPRARGTHR

SEQ ID NO: 7 - protein, 391 aa, Artificial
  Synthetic
  MISC_FEATURE: Heavy Chain Variable Domain
METGLTRPSERTRPVALPHELEPHEPHELESERVALTHRTHRGLYVALHISSERGLVALGLNLEVALGLNSERGLYALAGLVALLYSLYSPRGLYGLSERLEARGILESERCYSLYSGLYSERGLYTYRSERPHETHRALATYRTRPILEGLTRPVALARGGLNALAPRGLYLYSGLYLEGLTRPILEGLYGLILELEPRGLYSERASPSERTHRASNTYRASNGLLYSPHELYSGLYHISVALTHRILESERALAASPLYSSERILESERTHRALATYRLEGLNTRPSERSERLELYSALASERASPTHRALAVALTYRTYRCYSALAARGSERGLYTYRTYRGLYSERSERGLNTYRTRPGLYGLNGLYTHRLEVALTHRVALSERSER

SEQ ID NO: 8 - protein, 391 aa, Artificial; identical to SEQ ID NO: 7
  Synthetic
  MISC_FEATURE: Heavy Chain Variable Domain

SEQ ID NO: 9 - protein, 365 aa, Artificial
  Synthetic
  MISC_FEATURE: Light Chain Variable Domain
METSERVALPRTHRGLNVALLEGLYLELELELETRPLETHRASPALAARGCYSASPILEVALLETHRGLNSERPRALASERLEALAVALSERPRGLYGLNARGALATHRILETHRCYSARGALASERGLSERVALASPSERTYRGLYASNSERPHEMETHISTRPTYRGLNGLNLYSPRGLYGLNPRPRLYSLELEILETYRLETHRSERASNLEGLSERGLYVALPRASPARGPHESERGLYSERGLYSERGLYTHRASPPHETHRLETHRILEASNPRVALGLALAASNASPALAALATHRTYRTYRCYSGLNGLNASNALAGLASPPRARGTHRPHEGLYGLYGLYTHRLYSLEGLILELYS

SEQ ID NO: 10 - protein, 365 aa, Artificial; identical to SEQ ID NO: 9
  Synthetic
  MISC_FEATURE: Light Chain Variable Domain